European Patent Application EP 4 389 221 A2, published June 26, 2024. Title: Pan-Genotypic Agents Against Influenza Virus and Methods of Using the Same. Applicant: The Board of Trustees of the Leland Stanford Junior University. Application EP. The sequence listing filed with the application follows.

SEQUENCE LISTING (97 sequences)

SEQ ID NO: 1 - RNA, 196 nt, synthetic construct
  misc_feature 1..196: note = Synthetic polynucleotide
  source 1..196: mol_type = other RNA
agtagaaacaaggtcgtttttaaactattcgacactaattgatggccatccgaattcttttggtcgctgtctggctgtcagtaagtatgctagagtcccgttttcgtttcattaccaacaccacgtctccttgcccaattagcacattagccttttttattctttccatattgaatataattgacctgctttcgct

SEQ ID NO: 2 - RNA, 182 nt, synthetic construct
  misc_feature 1..182: note = Synthetic polynucleotide
  source 1..182: mol_type = other RNA
agtagaaacaaggtcgtttttaaactattcgacactaattgatcgccatccgaattcttttggtcgctgtctggctgtcagtaagtatgctagagtcccgttttcgtttcgcgagactgcgacattagatttcttagttcttttattctttccatattgaatataattgacctgctttcgct

SEQ ID NO: 3 - RNA, 197 nt, synthetic construct
  misc_feature 1..197: note = Synthetic polynucleotide
  source 1..197: mol_type = other RNA
agtagaaacaggtcgtttttaaactattcgacactaattgatggccatccgaattcttttggtcgctgtctggctgtctgtaagtatgctagagtcccgttttcgtttcggactctcaaaaacgtgcgagactgcgacattagatttcttagttcttttattctttccatattgaatataattgacctgctttcgct

SEQ ID NO: 4 - RNA, 158 nt, synthetic construct
  misc_feature 1..158: note = Synthetic polynucleotide
  source 1..158: mol_type = other RNA
agtagaaacaaggtcgtttttaaactattcgacactaattgatgatggccatccgaattcttttggtcgctgtctggctgtcagtaagtatgctagagtcccgtttccgtttcattaccaacaccacgtctcttgaatataattgacctgctttcgct

SEQ ID NO: 5 - RNA, 178 nt, synthetic construct
  misc_feature 1..178: note = Synthetic polynucleotide
  source 1..178: mol_type = other RNA
agtagaaacaaggtcgtttttaaataattcgacactaattgatggccatccgaattcttttggtcgctgtctggctgtcagtaagtatgctagagtcccgttttcgtttcattaccaacaccacgtctccttgcccttttattctctccatattgaatatatttgacctgctttcgct

SEQ ID NO: 6 - RNA, 289 nt, synthetic construct
  misc_feature 1..289: note = Synthetic polynucleotide
  source 1..289: mol_type = other RNA
agtagaaacaaggtcgtttttaaactattcgacactaattgatggccatccgaattcttttggtcgctgtctggctgtcagtaagtatgctagagtcccgttttcgtttcattaccaacactacgtccccttgcccaattagcacattagccttctctccttttgcaagattgctcagttcattgatgctaatgctgggccatatctcttgtcttctttgcccaaaatgagaaatcctctcaggacagcatattctctccatattgaatataattgacctgctttcgct

SEQ ID NO: 7 - RNA, 177 nt, synthetic construct
  misc_feature 1..177: note = Synthetic polynucleotide
  source 1..177: mol_type = other RNA
agtagaaacaaggtcgtttttaaactattcgacactaattgatggccatccgaattcttttggtcgctgtctggctgtcagtaagtatgctagagtcccgtttcgtttcattaccaacaccacgtctccttgcccttttattctttccatattgaatataattgacctgctttcgct

SEQ ID NO: 8 - RNA, 197 nt, synthetic construct
  misc_feature 1..197: note = Synthetic polynucleotide
  source 1..197: mol_type = other RNA
agtagaaacaaggtcgtttttaaactattcgacactaattgatggccatccgaattcttttggtcgctgtctggctgtcagttaatatgctagagtcccgttttcgtttcattaccaacaccacgtctccttgcccaattagcacgtcgataggttttttattctttccatattgaatataatgacctgctttcgct

SEQ ID NO: 9 - RNA, 198 nt, synthetic construct
  misc_feature 1..198: note = Synthetic polynucleotide
  source 1..198: mol_type = other RNA
agtagaaacaaggtcgtttttaaactattcgacactaattgatggccatccgaattcttttggtcgctgtctggctgtctgtaagtatgctagagtcccgttttcgtttcggactctcaaaaacgtgcgagactgcgacattagatttcttagttcttttattctttccatattgaatataattgacctgctttcgct

SEQ ID NO: 10 - RNA, 178 nt, synthetic construct
  misc_feature 1..178: note = Synthetic polynucleotide
  source 1..178: mol_type = other RNA
agtagaaacaaggtcgtttttaaactattcgacatctaattgatggccatccgaattcttttggtcgctgtctggctgtcagtaagtatgctagagtcccgttttcgtttgactgcgacattagatttcttagttcttttattctttccatattgaatataattgacctgctttcgct

SEQ ID NO: 11 - RNA, 182 nt, synthetic construct; identical to SEQ ID NO: 2
  misc_feature 1..182: note = Synthetic polynucleotide
  source 1..182: mol_type = other RNA

SEQ ID NO: 12 - RNA, 59 nt, synthetic construct
  misc_feature 1..59: note = Synthetic polynucleotide
  source 1..59: mol_type = other RNA
cgacactaattgatggccatccgaattcttttggtcgctgtctggctgtcagtaagtat

SEQ ID NO: 13 - RNA, 59 nt, synthetic construct; identical to SEQ ID NO: 12
  misc_feature 1..59: note = Synthetic polynucleotide
  source 1..59: mol_type = other RNA

SEQ ID NO: 14 - DNA, 108 bp, synthetic construct
  misc_feature 1..108: note = Synthetic polynucleotide
  source 1..108: mol_type = other DNA
attgggcaaggagacgtggtgttggtaatgaaacggaaacggaactctagcatacttactgacagccagacagcgaccaaaagaattcggatggccatcaattagtgt

SEQ ID NO: 15 - DNA, 108 bp, synthetic construct
  misc_feature 1..108: note = Synthetic polynucleotide
  source 1..108: mol_type = other DNA
attgggcaaggagacgtcgtgttggtaatgaaacggaaacggaactctagcatattaacagacagccaaacagcgacgaaaagaattcggatggcgatcaattgatgt

SEQ ID NO: 16 - DNA, 23 bp, synthetic construct
  misc_feature 1..23: note = Synthetic polynucleotide
  source 1..23: mol_type = other DNA
tacttactgacagtcagacagcg

SEQ ID NO: 17 - DNA, 23 bp, synthetic construct
  misc_feature 1..23: note = Synthetic polynucleotide
  source 1..23: mol_type = other DNA
cgctgtctgactgtcagtaagta

SEQ ID NO: 18 - DNA, 23 bp, synthetic construct
  misc_feature 1..23: note = Synthetic polynucleotide
  source 1..23: mol_type = other DNA
tacttactgactcgcagacagcg

SEQ ID NO: 19 - DNA, 23 bp, synthetic construct
  misc_feature 1..23: note = Synthetic polynucleotide
  source 1..23: mol_type = other DNA
cgctgtctgcgagtcagtaagta

SEQ ID NO: 20 - DNA, 30 bp, synthetic construct
  misc_feature 1..30: note = Synthetic polynucleotide
  source 1..30: mol_type = other DNA
tgacagccagactgcgaccaaaagaattcg

SEQ ID NO: 21 - DNA, 30 bp, synthetic construct
  misc_feature 1..30: note = Synthetic polynucleotide
  source 1..30: mol_type = other DNA
cgaattcttttggtcgcagtctggctgtca

SEQ ID NO: 22 - DNA, 24 bp, synthetic construct
  misc_feature 1..24: note = Synthetic polynucleotide
  source 1..24: mol_type = other DNA
agcgaccaaaagcattcggatggc

SEQ ID NO: 23 - DNA, 24 bp, synthetic construct
  misc_feature 1..24: note = Synthetic polynucleotide
  source 1..24: mol_type = other DNA
gccatccgaatgcttttggtcgct

SEQ ID NO: 24 - RNA, 175 nt, synthetic construct
  misc_feature 1..175: note = Synthetic polynucleotide
  source 1..175: mol_type = other RNA
agtagaaacaaggtcgtttttaaactattcgacactaattgatggccatccgaattcttttggtcgctgtcggctgtcagtaagtatgctagagtcccgttttcgtttcattaccaacacgacgtctccttgcttttattctttccatattgaatataattgacctgctttcgct

SEQ ID NO: 25 - RNA, 151 nt, synthetic construct
  misc_feature 1..151: note = Synthetic polynucleotide
  source 1..151: mol_type = other RNA
agtagaaacaaggtcgtttttaaactattcgacactaattgatggccatccgaattcttttcgtcgctgtctggctgtcagtaagtatgctagagtcccgttttcgtttctttattctttccatattgaatataattgacctgctttcgct

SEQ ID NO: 26 - RNA, 148 nt, synthetic construct
  misc_feature 1..148: note = Synthetic polynucleotide
  source 1..148: mol_type = other RNA
agtgaaacaaggtcgtttttaaactattcgacactaattgatggccatccgaattcttttggtcgctgtttggctgtcagtaagtatgctagagtcccgttttagtttttattctttccatattgaatataattgacctgctttcgct

SEQ ID NO: 27 - RNA, 59 nt, synthetic construct; identical to SEQ ID NO: 12
  misc_feature 1..59: note = Synthetic polynucleotide
  source 1..59: mol_type = other RNA

SEQ ID NO: 28 - DNA, 29 bp, synthetic construct
  misc_feature 1..29: note = Synthetic polynucleotide
  source 1..29: mol_type = other DNA
agaattcggatgcccatcaattagtgtcg

SEQ ID NO: 29 - DNA, 29 bp, synthetic construct
  misc_feature 1..29: note = Synthetic polynucleotide
  source 1..29: mol_type = other DNA
cgacactaattgatgggcatccgaattct

SEQ ID NO: 30 - DNA, 23 bp, synthetic construct
  misc_feature 1..23: note = Synthetic polynucleotide
  source 1..23: mol_type = other DNA
tacttactgacaggcagacagcg

SEQ ID NO: 31 - DNA, 23 bp, synthetic construct
  misc_feature 1..23: note = Synthetic polynucleotide
  source 1..23: mol_type = other DNA
cgctgtctgcctgtcagtaagta

SEQ ID NO: 32 - DNA, 25 bp, synthetic construct
  misc_feature 1..25: note = Synthetic polynucleotide
  source 1..25: mol_type = other DNA
ttcggatgggcatcaattagtgtcg

SEQ ID NO: 33 - DNA, 25 bp, synthetic construct
  misc_feature 1..25: note = Synthetic polynucleotide
  source 1..25: mol_type = other DNA
cgacactaattgatgcccatccgaa

SEQ ID NO: 34 - DNA, 24 bp, synthetic construct
  misc_feature 1..24: note = Synthetic polynucleotide
  source 1..24: mol_type = other DNA
atacttactgacacccagacagcg

SEQ ID NO: 35 - DNA, 24 bp, synthetic construct
  misc_feature 1..24: note = Synthetic polynucleotide
  source 1..24: mol_type = other DNA
cgctgtctgggtgtcagtaagtat

SEQ ID NO: 36 - DNA, 24 bp, synthetic construct
  misc_feature 1..24: note = Synthetic polynucleotide
  source 1..24: mol_type = other DNA
tcggatggccatgaattagtgtcg

SEQ ID NO: 37 - DNA, 24 bp, synthetic construct
  misc_feature 1..24: note = Synthetic polynucleotide
  source 1..24: mol_type = other DNA
cgacactaattcatggccatccga

SEQ ID NO: 38 - DNA, 26 bp, synthetic construct
  misc_feature 1..26: note = Synthetic polynucleotide
  source 1..26: mol_type = other DNA
agcatacttactcacagccagacagc

SEQ ID NO: 39 - DNA, 26 bp, synthetic construct
  misc_feature 1..26: note = Synthetic polynucleotide
  source 1..26: mol_type = other DNA
gctgtctggctgtgagtaagtatgct

SEQ ID NO: 40 - DNA, 34 bp, synthetic construct
  misc_feature 1..34: note = Synthetic polynucleotide
  source 1..34: mol_type = other DNA
ccaaaagaattaggatggccatcaattagtgtcg

SEQ ID NO: 41 - DNA, 34 bp, synthetic construct
  misc_feature 1..34: note = Synthetic polynucleotide
  source 1..34: mol_type = other DNA
cgacactaattgatggccatcctaattcttttgg

SEQ ID NO: 42 - DNA, 29 bp, synthetic construct
  misc_feature 1..29: note = Synthetic polynucleotide
  source 1..29: mol_type = other DNA
gacagccagacagctaccaaaagaattcg

SEQ ID NO: 43 - DNA, 29 bp, synthetic construct
  misc_feature 1..29: note = Synthetic polynucleotide
  source 1..29: mol_type = other DNA
cgaattcttttggtagctgtctggctgtc

SEQ ID NO: 44 - RNA, 71 nt, synthetic construct
  misc_feature 1..71: note = Synthetic polynucleotide
  source 1..71: mol_type = other RNA
tcgacactaattgatggccatccgaattcttttggtcgctgtctggctgtcagtaagtatgctagccttgc

SEQ ID NO: 45 - DNA, 11 bp, synthetic construct
  misc_feature 1..11: note = Synthetic polynucleotide
  source 1..11: mol_type = other DNA
accaaaagaat

SEQ ID NO: 46 - DNA, 11 bp, synthetic construct
  misc_feature 1..11: note = Synthetic polynucleotide
  source 1..11: mol_type = other DNA
tggccatcaat

SEQ ID NO: 47 - DNA, 11 bp, synthetic construct
  misc_feature 1..11: note = Synthetic polynucleotide
  source 1..11: mol_type = other DNA
tagcatactta

SEQ ID NO: 48-49 - skipped (2 entries)

SEQ ID NO: 50 - DNA, 15 bp, synthetic construct
  misc_feature 1..15: note = Synthetic polynucleotide
  source 1..15: mol_type = other DNA
cagacacgaccaaaa

SEQ ID NO: 51 - DNA, 15 bp, synthetic construct
  misc_feature 1..15: note = Synthetic polynucleotide
  source 1..15: mol_type = other DNA
tacttactgacagcc

SEQ ID NO: 52 - DNA, 15 bp, synthetic construct
  misc_feature 1..15: note = Synthetic polynucleotide
  source 1..15: mol_type = other DNA
agacacgaccaaaag

SEQ ID NO: 53 - DNA, 11 bp, synthetic construct
  misc_feature 1..11: note = Synthetic polynucleotide
  source 1..11: mol_type = other DNA
accaaaagaat

SEQ ID NO: 54 - DNA, 11 bp, synthetic construct
  misc_feature 1..11: note = Synthetic polynucleotide
  source 1..11: mol_type = other DNA
tggccatcaat

SEQ ID NO: 55 - DNA, 11 bp, synthetic construct
  misc_feature 1..11: note = Synthetic polynucleotide
  source 1..11: mol_type = other DNA
tagcatactta

SEQ ID NO: 56 - DNA, 15 bp, synthetic construct
  misc_feature 1..15: note = Synthetic polynucleotide
  source 1..15: mol_type = other DNA
cgaccaaaagaattc

SEQ ID NO: 57 - DNA, 15 bp, synthetic construct
  misc_feature 1..15: note = Synthetic polynucleotide
  source 1..15: mol_type = other DNA
cgaccaaaagaattc

SEQ ID NO: 58 - DNA, 15 bp, synthetic construct
  misc_feature 1..15: note = Synthetic polynucleotide
  source 1..15: mol_type = other DNA
gatggccatcaatta

SEQ ID NO: 59 - DNA, 15 bp, synthetic construct
  misc_feature 1..15: note = Synthetic polynucleotide
  source 1..15: mol_type = other DNA
gatggccatcaatta

SEQ ID NO: 60 - DNA, 15 bp, synthetic construct
  misc_feature 1..15: note = Synthetic polynucleotide
  source 1..15: mol_type = other DNA
tctagcatacttact

SEQ ID NO: 61 - DNA, 15 bp, synthetic construct
  misc_feature 1..15: note = Synthetic polynucleotide
  source 1..15: mol_type = other DNA
tctagcatacttact

SEQ ID NO: 62 - DNA, 15 bp, synthetic construct
  misc_feature 1..15: note = Synthetic polynucleotide
  source 1..15: mol_type = other DNA
gaattcggatggcca

SEQ ID NO: 63 - DNA, 15 bp, synthetic construct
  misc_feature 1..15: note = Synthetic polynucleotide
  source 1..15: mol_type = other DNA
ggccatcaattagtg

SEQ ID NO: 64 - DNA, 15 bp, synthetic construct
  misc_feature 1..15: note = Synthetic polynucleotide
  source 1..15: mol_type = other DNA
ttcggatggccatca

SEQ ID NO: 65 - DNA, 13 bp, synthetic construct
  misc_feature 1..13: note = Synthetic polynucleotide
  source 1..13: mol_type = other DNA
agccagacagcga

SEQ ID NO: 66 - DNA, 15 bp, synthetic construct
  misc_feature 1..15: note = Synthetic polynucleotide
  source 1..15: mol_type = other DNA
gacagccagacagca

SEQ ID NO: 67 - DNA, 11 bp, synthetic construct
  misc_feature 1..11: note = Synthetic polynucleotide
  misc_feature 1: note = LNA
  misc_feature 4: note = LNA
  misc_feature 7..8: note = LNA
  misc_feature 11: note = LNA
  source 1..11: mol_type = other DNA
accaaaagaat

SEQ ID NO: 68 - DNA, 11 bp, synthetic construct
  misc_feature 1..11: note = Synthetic polynucleotide
  misc_feature 1: note = LNA
  misc_feature 4: note = LNA
  misc_feature 6..7: note = LNA
  misc_feature 11: note = LNA
  source 1..11: mol_type = other DNA
tggccatcaat

SEQ ID NO: 69 - DNA, 11 bp, synthetic construct
  misc_feature 1..11: note = Synthetic polynucleotide
  misc_feature 1: note = LNA
  misc_feature 4..5: note = LNA
  misc_feature 7: note = LNA
  misc_feature 11: note = LNA
  source 1..11: mol_type = other DNA
tagcatactta

SEQ ID NO: 70-71 - skipped (2 entries)

SEQ ID NO: 72 - DNA, 15 bp, synthetic construct
  misc_feature 1..15: note = Synthetic polynucleotide
  misc_feature 1: note = LNA
  misc_feature 5: note = LNA
  misc_feature 7..8: note = LNA
  misc_feature 10..11: note = LNA
  misc_feature 14..15: note = LNA
  source 1..15: mol_type = other DNA
cagacacgaccaaaa

SEQ ID NO: 73 - DNA, 15 bp, synthetic construct
  misc_feature 1..15: note = Synthetic polynucleotide
  misc_feature 1..2: note = LNA
  misc_feature 4: note = LNA
  misc_feature 7..8: note = LNA
  misc_feature 11: note = LNA
  misc_feature 14..15: note = LNA
  source 1..15: mol_type = other DNA
tacttactgacagcc

SEQ ID NO: 74 - DNA, 15 bp, synthetic construct
  misc_feature 1..15: note = Synthetic polynucleotide
  misc_feature 1..4: note = LNA
  misc_feature 12..15: note = LNA
  source 1..15: mol_type = other DNA
agacacgaccaaaag

SEQ ID NO: 75 - DNA, 15 bp, synthetic construct
  misc_feature 1..15: note = Synthetic polynucleotide
  misc_feature 1..4: note = LNA
  misc_feature 13..15: note = LNA
  source 1..15: mol_type = other DNA
tacttactgacagcc

SEQ ID NO: 76 - DNA, 15 bp, synthetic construct
  misc_feature 1..15: note = Synthetic polynucleotide
  misc_feature 1..3: note = LNA
  misc_feature 12..15: note = LNA
  source 1..15: mol_type = other DNA
tacttactgacagcc

SEQ ID NO: 77 - DNA, 11 bp, synthetic construct
  misc_feature 1..11: note = Synthetic polynucleotide
  misc_feature 1..3: note = LNA
  misc_feature 9..11: note = LNA
  source 1..11: mol_type = other DNA
accaaaagaat

SEQ ID NO: 78 - DNA, 11 bp, synthetic construct
  misc_feature 1..11: note = Synthetic polynucleotide
  misc_feature 1..3: note = LNA
  misc_feature 9..11: note = LNA
  source 1..11: mol_type = other DNA
tggccatcaat

SEQ ID NO: 79 - DNA, 11 bp, synthetic construct
  misc_feature 1..11: note = Synthetic polynucleotide
  misc_feature 1..3: note = LNA
  misc_feature 9..11: note = LNA
  source 1..11: mol_type = other DNA
tagcatactta

SEQ ID NO: 80 - DNA, 15 bp, synthetic construct
  misc_feature 1..15: note = Synthetic polynucleotide
  misc_feature 1: note = LNA
  misc_feature 5..6: note = LNA
  misc_feature 9..10: note = LNA
  misc_feature 15: note = LNA
  source 1..15: mol_type = other DNA
cgaccaaaagaattc

SEQ ID NO: 81 - DNA, 15 bp, synthetic construct
  misc_feature 1..15: note = Synthetic polynucleotide
  misc_feature 1..4: note = LNA
  misc_feature 12..15: note = LNA
  source 1..15: mol_type = other DNA
cgaccaaaagaattc

SEQ ID NO: 82 - DNA, 15 bp, synthetic construct
  misc_feature 1..15: note = Synthetic polynucleotide
  misc_feature 1: note = LNA
  misc_feature 3..4: note = LNA
  misc_feature 6: note = LNA
  misc_feature 8..9: note = LNA
  misc_feature 12: note = LNA
  misc_feature 15: note = LNA
  source 1..15: mol_type = other DNA
gatggccatcaatta

SEQ ID NO: 83 - DNA, 15 bp, synthetic construct
  misc_feature 1..15: note = Synthetic polynucleotide
  misc_feature 1..4: note = LNA
  misc_feature 12..15: note = LNA
  source 1..15: mol_type = other DNA
gatggccatcaatta

SEQ ID NO: 84 - DNA, 15 bp, synthetic construct
  misc_feature 1..15: note = Synthetic polynucleotide
  misc_feature 1: note = LNA
  misc_feature 3..4: note = LNA
  misc_feature 6: note = LNA
  misc_feature 8..9: note = LNA
  misc_feature 12: note = LNA
  misc_feature 15: note = LNA
  source 1..15: mol_type = other DNA
tctagcatacttact

SEQ ID NO: 85 - DNA, 15 bp, synthetic construct
  misc_feature 1..15: note = Synthetic polynucleotide
  misc_feature 1..4: note = LNA
  misc_feature 12..15: note = LNA
  source 1..15: mol_type = other DNA
tctagcatacttact

SEQ ID NO: 86 - DNA, 15 bp, synthetic construct
  misc_feature 1..15: note = Synthetic polynucleotide
  misc_feature 1..3: note = LNA
  misc_feature 12..15: note = LNA
  source 1..15: mol_type = other DNA
gaattcggatggcca

SEQ ID NO: 87 - DNA, 15 bp, synthetic construct
  misc_feature 1..15: note = Synthetic polynucleotide
  misc_feature 1..4: note = LNA
  misc_feature 13..15: note = LNA
  source 1..15: mol_type = other DNA
ggccatcaattagtg

SEQ ID NO: 88 - DNA, 15 bp, synthetic construct
  misc_feature 1..15: note = Synthetic polynucleotide
  misc_feature 1..4: note = LNA
  misc_feature 13..15: note = LNA
  source 1..15: mol_type = other DNA
ttcggatggccatca

SEQ ID NO: 89 - DNA, 13 bp, synthetic construct
  misc_feature 1..13: note = Synthetic polynucleotide
  misc_feature 1..4: note = LNA
  misc_feature 11..13: note = LNA
  source 1..13: mol_type = other DNA
agccagacagcga

SEQ ID NO: 90 - DNA, 15 bp, synthetic construct
  misc_feature 1..15: note = Synthetic polynucleotide
  misc_feature 1..4: note = LNA
  misc_feature 13..15: note = LNA
  source 1..15: mol_type = other DNA
gacagccagacagca

SEQ ID NO: 91 - DNA, 15 bp, synthetic construct
  misc_feature 1..15: note = Synthetic polynucleotide
  source 1..15: mol_type = other DNA
tacttactgacagtc

SEQ ID NO: 92 - DNA, 15 bp, synthetic construct
  misc_feature 1..15: note = Synthetic polynucleotide
  source 1..15: mol_type = other DNA
tacttaccgacagcc

SEQ ID NO: 93 - DNA, 16 bp, synthetic construct
  misc_feature 1..16: note = Synthetic polynucleotide
  source 1..16: mol_type = other DNA
ggatttcggatggcca

SEQ ID NO: 94 - DNA, 15 bp, synthetic construct
  misc_feature 1..15: note = Synthetic polynucleotide
  misc_feature 1..4: note = LNA
  misc_feature 13..15: note = LNA
  source 1..15: mol_type = other DNA
tacttactgacagtc

SEQ ID NO: 95 - DNA, 15 bp, synthetic construct
  misc_feature 1..15: note = Synthetic polynucleotide
  misc_feature 1..4: note = LNA
  misc_feature 13..15: note = LNA
  source 1..15: mol_type = other DNA
tacttaccgacagcc

SEQ ID NO: 96 - DNA, 16 bp, synthetic construct
  misc_feature 1..16: note = Synthetic polynucleotide
  misc_feature 1..4: note = LNA
  misc_feature 14..16: note = LNA
  source 1..16: mol_type = other DNA
ggatttcggatggcca

SEQ ID NO: 97 - DNA, 26 bp, synthetic construct
  misc_feature 1..26: note = Synthetic polynucleotide
  source 1..26: mol_type = other DNA
agggctcttcggccagcraaagcagg